European Patent Application EP 4 733 762 A1, published April 29, 2026. Title: Method of capturing and detecting extracellular vesicles originated from cancer cells, and kit. Applicant: TORAY INDUSTRIES, INC. The sequence listing filed with the application follows.

SEQUENCE LISTING (67 sequences)

SEQ ID NO: 1 - protein, 640 aa, Plasmodium falciparum
NYIKGDPYFAEYATKLSFILNPSDANNPSGETANHNDEACNCNESGISSVGQAQTSGPSSNKTCITHSSIKTNKKKECKDVKLGVRENDKDLKICVIEDTSLSGVDNCCCQDLLGILQENCSDNKRGSSSNDSCDNKNQDECQKKLEKVFASLTNGYKCDKCKSGTSRSKKKWIWKKSSGNEEGLQEEYANTIGLPPRTQSLYLGNLPKLENVCEDVKDINFDTKEKFLAGCLIVSFHEGKNLKKRYPQNKNSGNKENLCKALEYSFADYGDLIKGTSIWDNEYTKDLELNLQNNFGKLFGKYIKKNNTAEQDTSYSSLDELRESWWNTNKKYIWTAMKHGAEMNITTCNADGSVTGSGSSCDDIPTIDLIPQYLRFLQEWVENFCEQRQAKVKDVITNCKSCKESGNKCKTECKTKCKDECEKYKKFIEACGTAGGGIGTAGSPWSKRWDQIYKRYSKHIEDAKRNRKAGTKNCGTSSTTNAAASTDENKCVQSDIDSFFKHLIDIGLTTPSSYLSNVLDDNICGADKAPWTTYTTYTTTEKCNKERDKSKSQSSDTLVVVNVPSPLGNTPYRYKYACQCKIPTNEETCDDRKEYMNQWSCGSARTMKRGYKNDNYELCKYNGVDVKPTTVRSNSSKLD

SEQ ID NO: 2 - DNA, 1920 bp, Plasmodium falciparum
  source 1..1920: mol_type = genomic DNA
aactacatcaagggcgacccctatttcgctgagtacgctacaaaactgagcttcatcctgaaccccagcgacgccaacaaccccagcggcgagacagccaaccacaacgacgaggcctgcaactgcaacgagagcggcatcagcagcgtgggccaggctcagacatccggccctagcagcaacaagacctgtatcacccacagctccatcaagaccaacaagaaaaaagaatgcaaggacgtgaagctgggcgtgcgggagaacgacaaggatctgaagatctgcgtgatcgaggacaccagcctgagcggcgtggacaactgctgctgccaggatctgctgggcatcctgcaggaaaactgcagcgacaacaagcggggcagcagctccaacgacagctgcgacaataagaaccaggacgagtgccagaaaaagctggaaaaggtgttcgccagcctgaccaacggctacaagtgcgataagtgcaagagcggcacctcccggtccaagaagaagtggatctggaagaagtccagcggcaacgaggaaggcctgcaggaagagtacgccaacaccatcggcctgccccccaggacccagagcctgtacctgggcaatctgcccaaactggaaaacgtgtgcgaggatgtgaaggacatcaacttcgacaccaaagagaagtttctggccggctgcctgatcgtgtccttccacgagggcaagaatctgaagaagcgctacccccagaataagaacagcggcaacaaagaaaacctgtgcaaggctctggaatacagcttcgccgactacggcgacctgatcaagggcacctccatctgggacaacgagtacacaaaggacctggaactgaatctgcagaacaacttcggcaagctgttcggcaagtacatcaagaagaacaataccgccgagcaggacacctcctacagctccctggacgagctgcgcgagtcttggtggaataccaataagaagtacatctggaccgccatgaagcacggcgccgagatgaacatcaccacctgtaacgccgacggctccgtgaccggcagcggctccagctgcgacgacatccccaccatcgacctgatcccccagtacctgagatttctgcaggaatgggtcgagaacttctgcgagcagcggcaggccaaagtgaaggacgtgatcaccaactgcaagagctgcaaagaatccggcaacaaatgcaagaccgagtgcaaaaccaagtgcaaggatgagtgcgagaagtacaagaagttcatcgaggcctgcggcacagccggcggaggcatcggaacagccggcagcccctggtccaagagatgggaccagatctacaagcggtacagcaagcacatcgaggacgccaagcggaaccggaaggccggcaccaagaactgcggcaccagctccaccaccaacgccgctgccagcaccgacgagaataagtgcgtgcagagcgacatcgacagctttttcaagcacctgatcgatatcggcctgaccacccccagcagctacctgagcaacgtgctggacgacaacatctgtggcgccgacaaggccccctggacaacctatacaacatacactacaaccgagaagtgcaacaaagagcgggacaagagcaagagccagagcagcgacaccctggtggtggtgaacgtgcccagccccctgggcaacacaccctaccggtacaagtacgcctgccagtgcaagatccccaccaacgaggaaacatgcgacgaccggaaagaatacatgaaccagtggtcctgcgggagcgctcggaccatgaagagagggtataagaacgataactacgaactgtgcaagtacaacggcgtggatgtgaagcccaccaccgtgcggagcaactccagcaagctggac

SEQ ID NO: 3 - protein, 28 aa, synthetic construct
WSHPQFEKGGGSGGGSGGSAWSHPQFEK

SEQ ID NO: 4 - protein, 12 aa, synthetic construct
GSAGSAAGSGEF

SEQ ID NO: 5 - protein, 22 aa, synthetic construct
DYKDHDGDYKDHDIDYKDDDDK

SEQ ID NO: 6 - protein, 710 aa, Plasmodium falciparum
MSAWSHPQFEKGGGSGGGSGGSAWSHPQFEKGSAGSAAGSGEFNYIKGDPYFAEYATKLSFILNPSDANNPSGETANHNDEACNCNESGISSVGQAQTSGPSSNKTCITHSSIKTNKKKECKDVKLGVRENDKDLKICVIEDTSLSGVDNCCCQDLLGILQENCSDNKRGSSSNDSCDNKNQDECQKKLEKVFASLTNGYKCDKCKSGTSRSKKKWIWKKSSGNEEGLQEEYANTIGLPPRTQSLYLGNLPKLENVCEDVKDINFDTKEKFLAGCLIVSFHEGKNLKKRYPQNKNSGNKENLCKALEYSFADYGDLIKGTSIWDNEYTKDLELNLQNNFGKLFGKYIKKNNTAEQDTSYSSLDELRESWWNTNKKYIWTAMKHGAEMNITTCNADGSVTGSGSSCDDIPTIDLIPQYLRFLQEWVENFCEQRQAKVKDVITNCKSCKESGNKCKTECKTKCKDECEKYKKFIEACGTAGGGIGTAGSPWSKRWDQIYKRYSKHIEDAKRNRKAGTKNCGTSSTTNAAASTDENKCVQSDIDSFFKHLIDIGLTTPSSYLSNVLDDNICGADKAPWTTYTTYTTTEKCNKERDKSKSQSSDTLVVVNVPSPLGNTPYRYKYACQCKIPTNEETCDDRKEYMNQWSCGSARTMKRGYKNDNYELCKYNGVDVKPTTVRSNSSKLDGGADYKDHDGDYKDHDIDYKDDDDKLE

SEQ ID NO: 7 - DNA, 2133 bp, Plasmodium falciparum
  source 1..2133: mol_type = other DNA
catatgagcgcttggagccacccgcagttcgagaaaggtggaggttccggaggtggatcgggaggttcggcgtggagccacccgcagttcgaaaaaggatccgctggctccgctgctggttctggcgagttcaactatatcaagggtgacccctatttcgctgaatacgcaaccaagctgtcattcatcctcaatccgtcagatgcaaacaatccgagtggtgagacagcaaaccataacgatgaagcatgtaattgcaatgaatctggaatttcttcggtcggccaggcccagacgtcagggccgtcaagtaataagacatgcattacccacagcagtatcaaaacaaacaagaagaaggaatgtaaggacgtcaagctcggagtgcgcgaaaacgataaagaccttaagatttgcgttatcgaggatacctcgctgtccggtgtagataattgctgttgtcaggatttgctgggcattcttcaggagaactgctctgacaataagcgtggtagcagtagcaacgattcttgtgacaataagaaccaagatgaatgccagaagaagttagaaaaggtcttcgcgagtcttacgaatggctacaaatgtgacaagtgcaagtcagggaccagtcgctccaagaagaagtggatttggaagaaatctagcggaaatgaagaaggcttgcaggaggagtatgcaaacacaattggcctccctcctcgcactcagtcgctttacctggggaacttgccgaagcttgagaatgtttgcgaagatgtgaaagacatcaactttgacaccaaagagaagttcctggctggttgcttaatcgtgtccttccacgagggaaagaacctgaagaaacgttacccgcagaacaagaattctggaaacaaggagaacttgtgtaaggccttggaatatagtttcgccgattacggggacttaatcaagggaactagcatttgggacaatgagtacacaaaggatcttgagctcaaccttcaaaacaacttcggtaagctctttggaaagtatattaagaagaataatactgccgaacaagatacgtcttattcttctttggatgagctgcgcgaatcttggtggaacactaataagaaatacatctggacggcgatgaaacatggggctgagatgaacatcactacatgtaacgcggacggtagcgtcactgggtcgggatcgagttgtgatgacatcccaacgattgaccttattccacagtacttgcgcttcctccaagaatgggtcgagaatttctgcgagcagcgccaagccaaagttaaggacgttatcacaaattgtaagtcttgtaaagaatcgggaaataagtgtaaaactgaatgcaagacgaagtgcaaggacgaatgtgagaagtataagaagttcattgaagcctgtgggacagctggcggtggtatcggtacagccgggtcgccatggtcgaaacgttgggaccagatttacaagcgttacagcaagcatatcgaagatgccaaacgcaatcgtaaggcaggaaccaagaattgcggtacgtcctcaaccactaatgcggccgcgtctactgatgaaaacaaatgcgttcaatcagatatcgatagcttcttcaagcatcttatcgacatcgggctcacaacacctagcagctatctgagtaacgtattagatgataacatttgtggagcagataaagcgccgtggaccacctatactacttataccaccacggaaaagtgtaacaaggaacgtgataagtctaagtcacaatcatccgataccttggtcgtcgtcaacgtccctagtcctctgggcaatacaccgtaccgttacaagtacgcatgccaatgtaaaatcccgaccaatgaagaaacatgcgacgaccgcaaggaatatatgaatcagtggtcgtgtggctcggctcgtactatgaagcgtggctataagaatgacaattatgaactctgcaagtataatggtgttgatgttaaaccgacaacggtacgttctaacagttcaaagctggatggtggcgccgactacaaagaccatgacggtgattataaagatcatgacatcgattacaaggatgacgatgacaagctcgag

SEQ ID NO: 8 - protein, 716 aa, Plasmodium falciparum
MSAWSHPQFEKGGGSGGGSGGSAWSHPQFEKGSAGSAAGSGEFNYIKGDPYFAEYATKLSFILNPSDANNPSGETANHNDEACNCNESGISSVGQAQTSGPSSNKTCITHSSIKTNKKKECKDVKLGVRENDKDLKICVIEDTSLSGVDNCCCQDLLGILQENCSDNKRGSSSNDSCDNKNQDECQKKLEKVFASLTNGYKCDKCKSGTSRSKKKWIWKKSSGNEEGLQEEYANTIGLPPRTQSLYLGNLPKLENVCEDVKDINFDTKEKFLAGCLIVSFHEGKNLKKRYPQNKNSGNKENLCKALEYSFADYGDLIKGTSIWDNEYTKDLELNLQNNFGKLFGKYIKKNNTAEQDTSYSSLDELRESWWNTNKKYIWTAMKHGAEMNITTCNADGSVTGSGSSCDDIPTIDLIPQYLRFLQEWVENFCEQRQAKVKDVITNCKSCKESGNKCKTECKTKCKDECEKYKKFIEACGTAGGGIGTAGSPWSKRWDQIYKRYSKHIEDAKRNRKAGTKNCGTSSTTNAAASTDENKCVQSDIDSFFKHLIDIGLTTPSSYLSNVLDDNICGADKAPWTTYTTYTTTEKCNKERDKSKSQSSDTLVVVNVPSPLGNTPYRYKYACQCKIPTNEETCDDRKEYMNQWSCGSARTMKRGYKNDNYELCKYNGVDVKPTTVRSNSSKLDGGADYKDHDGDYKDHDIDYKDDDDKLEHHHHHH

SEQ ID NO: 9 - protein, 632 aa, Plasmodium falciparum
NYIKDDPYSKEYVTKLSFIPNSSDANTSSEKIQKNNDEVCNPNESGISSVEQAQTSGPSSNKTCITHSSIKANKKKECKDVKLGVRENDKDLKICVIEDTSLSGVDNCCCQDLLGILQENCSDNKRGSSSNDSCDNKNQDECQKKLDEALESLHNGYKNQKCKSGTSTVNKKWIWKKSSGNKEGLQKEYANTIGLPPRTQSLYLGNLPKLENVSKGVTDIIYDTKEKFLAGCLIVSFHEGKNLKTSHEKKNDDNGKKLCKALEYSFADYGDLIKGTSIWDNEYTKDLELNLQKAFGKLFRKYIKKNISAEQDTSYSSLDELRESWWNTNKKYIWIAMKHGAGMNGTTCCGDGSSGENQTNSCDDIPTIDLIPQYLRFLQEWVEHFCEQRQAKVKDVITNCKSCKNTSGERKIGGTCNGECKTKCKNKCEAYKTFIEHCKGGDGTAGSSWVKRWDQIYKRYSKHIEDAKRNRKAGTKSCGTSTAENKCVQSDIDSFFKHLIDIGLTTPSSYLSIVLDENNCGEDKAPWTTYTTTKNCDIQKDKSKSQSSDTLVVVNVPSPLGNTPHGYKYACQCKIPTTEETCDDRKEYMNQWSCGSARTMKRGYKNDNYELCKYNGVDVKPTTVRSSSTKLD

SEQ ID NO: 10 - DNA, 2147 bp, Plasmodium falciparum
  source 1..2147: mol_type = genomic DNA
catatgagcgcttggagccacccgcagttcgagaaaggtggaggttccggaggtggatcgggaggttcggcgtggagccacccgcagttcgaaaaaggatccgctggctccgctgctggttctggcgagttcaactacatcaaggacgatccttatagcaaagagtatgtcaccaaactgagctttatcccgaattcatcagatgcaaatacgtcatcagagaaaatccagaagaacaacgacgaggtctgcaatcctaatgaaagtggtattagctcggtggaacaggctcagacatctggtccaagttcaaataaaacgtgtataacgcattcgagcattaaagccaacaagaagaaagagtgcaaggatgtaaaactgggcgtaagagaaaacgataaagacctgaaaatctgcgtgatagaagatactagtttaagtggagttgataattgctgctgccaggatttgctgggtattttacaagaaaattgtagcgataataaacggggttccagctctaatgattcctgtgataacaagaaccaggacgaatgccaaaagaaactggatgaagccttggaatctttgcataatggctataagaaccagaaatgcaaatccgggacgtcaacagtaaataagaaatggatttggaagaagtccagcggtaataaagaaggtttacagaaagagtatgcgaataccattggccttccgccacgaacacaaagtctttatctgggaaatctccccaaattggaaaatgttagcaaaggggtgaccgatattatttatgacacgaaagagaaattcctggcgggttgtttaattgtgtcctttcacgaaggcaagaaccttaaaacctcacatgaaaagaagaacgacgacaacgggaagaaactgtgtaaagccttagaatatagctttgccgattatggggatcttattaaagggacttcgatatgggataatgaatataccaaagacctggagctcaacttacagaaagcatttggcaaactgtttcgcaaatacattaagaagaacatcagcgcggagcaagatacatcatattcttctcttgacgagctgcgtgaatcttggtggaatactaataagaaatacatctggatcgccatgaagcatggtgcaggaatgaatggaacgacctgttgtggcgatggctcttcaggggaaaatcaaacaaatagttgtgatgatatcccgaccattgatttaatcccgcagtatctccgctttctgcaggaatgggttgaacatttctgtgaacagcgccaagcaaaagtaaaagatgttattacgaactgcaaatcctgcaagaacacgtctggtgaacgtaaaattggtggaacttgtaatggggaatgtaaaaccaaatgcaagaacaaatgcgaggcctataaaacgtttatagagcattgcaaaggcggcgatggtactgctggtagtagttgggtaaaacgttgggatcaaatatacaaacgctactcgaaacacatagaggatgcaaaacggaatcgcaaagctggtactaaatcttgtggtactagcactgctgaaaataaatgtgtgcagtccgatattgactcgttctttaaacacctgatagacattggcctgaccacaccatcaagttatctatctattgtgctggacgagaataactgtggcgaagataaagcgccatggactacatatacgaccaccaagaattgcgacattcagaaagacaaaagcaaatcgcagtcctctgatacactagttgttgttaatgtgccgagtcctttaggtaatacccctcatggatataaatacgcgtgtcaatgtaaaatcccgaccaccgaagaaacctgtgatgatcgtaaagagtatatgaaccagtggagctgtggcagtgcaagaactatgaaaaggggatataagaacgacaactacgaactttgcaaatacaatggcgtcgatgtcaaacccacaacagttcgtagttcatcaacaaaattggacggtggcgccgactacaaagaccatgacggtgattataaagatcatgacatcgattacaaggatgacgatgacaagggtggatctcaccaccaccaccaccactgatctagagcggccgc

SEQ ID NO: 11 - protein, 709 aa, Plasmodium falciparum
MSAWSHPQFEKGGGSGGGSGGSAWSHPQFEKGSAGSAAGSGEFNYIKDDPYSKEYVTKLSFIPNSSDANTSSEKIQKNNDEVCNPNESGISSVEQAQTSGPSSNKTCITHSSIKANKKKECKDVKLGVRENDKDLKICVIEDTSLSGVDNCCCQDLLGILQENCSDNKRGSSSNDSCDNKNQDECQKKLDEALESLHNGYKNQKCKSGTSTVNKKWIWKKSSGNKEGLQKEYANTIGLPPRTQSLYLGNLPKLENVSKGVTDIIYDTKEKFLAGCLIVSFHEGKNLKTSHEKKNDDNGKKLCKALEYSFADYGDLIKGTSIWDNEYTKDLELNLQKAFGKLFRKYIKKNISAEQDTSYSSLDELRESWWNTNKKYIWIAMKHGAGMNGTTCCGDGSSGENQTNSCDDIPTIDLIPQYLRFLQEWVEHFCEQRQAKVKDVITNCKSCKNTSGERKIGGTCNGECKTKCKNKCEAYKTFIEHCKGGDGTAGSSWVKRWDQIYKRYSKHIEDAKRNRKAGTKSCGTSTAENKCVQSDIDSFFKHLIDIGLTTPSSYLSIVLDENNCGEDKAPWTTYTTTKNCDIQKDKSKSQSSDTLVVVNVPSPLGNTPHGYKYACQCKIPTTEETCDDRKEYMNQWSCGSARTMKRGYKNDNYELCKYNGVDVKPTTVRSSSTKLDGGADYKDHDGDYKDHDIDYKDDDDKGGSHHHHHH

SEQ ID NO: 12 - protein, 620 aa, Plasmodium falciparum
SYVKNNPYSAEYGKLLIFDNTNAFKESITFNKNVCSCSGNEKLIISEGSSSSSSFGTSSSYQSSIITSKKRNECAQIKFSGNENNMNINICSTQDEKLLVKLEDLLKGFCNISGVNTGGVEVVSEENCEEQFKKLLPSLEKCTILTCKECNKTRCKPLKKVEEKWIWRKFPGNGEGLQKEYANTIGLPPRTQSLYLGNLPKLENVCEDVKDINFDTKEKFLAGCLIAAFHEGKNLKKRYPQNKNDDNGKKLCKALEYSFADNGDLIKGTSIWDNEYTKDLELNLQKAFGKLFGKYIKKNNTAEQHTSYSSLDELRESWWNTNKKYIWLAMKHGAEMNGTTCSCSGDSSNDMPTIDLIPQYLRFLQEWVEHFCKQRQAKVKPVIENCKSCKESGGTCNGECKTECKNKCEAYKNFIEDCKRGDGTAGSSWSKRWDQIYKRYSKHIEDAKRNRKAGTKNCGPSSITNAAASTDESKCVQSDIDSFFKHLIDIGLTTPSSYLSIVLDENNCGDDKAPWTTYTTTKNCDIQKKTPKPQQSDTSVVVNVPSPLGNTPYRYKYACQCKIPTTEESCDDRKEYMNQWSCGSAQTVRGRSGKDYYELCKYNGVQIKPTTVRSNSTKLD

SEQ ID NO: 13 - protein, 632 aa, Plasmodium falciparum
NYIKGDPYFAEYATKLSFILNSSDANNPSEKIQKNNDEVCNCNESGIASVEQEQISDPSSNKTCITHSSIKANKKKVCKHVKLGVRENDKDLRVCVIEHTSLSGVENCCCQDFLRILQENCSDNKSGSSSNGSCNNKNQEACEKNLEKVLASLTNCYKCDKCKSEQSKKNNKNWIWKKSSGKEGGLQKEYANTIGLPPRTQSLCLVVCLDEKGKKTQELKNIRTNSELLKEWIIAAFHEGKNLKPSHEKKNDDNGKKLCKALEYSFADYGDLIKGTSIWDNEYTKDLELNLQKIFGKLFRKYIKKNNTAEQDTSYSSLDELRESWWNTNKKYIWLAMKHGAGMNSTTCCGDGSVTGSGSSCDDIPTIDLIPQYLRFLQEWVEHFCKQRQEKVKPVIENCKSCKESGGTCNGECKTECKNKCEVYKKFIEDCKGGDGTAGSSWVKRWDQIYKRYSKYIEDAKRNRKAGTKNCGPSSTTNAAENKCVQSDIDSFFKHLIDIGLTTPSSYLSIVLDDNICGADKAPWTTYTTYTTTEKCNKETDKSKLQQCNTAVVVNVPSPLGNTPHGYKYACQCKIPTNEETCDDRKEYMNQWSCGSARTMKRGYKNDNYELCKYNGVDVKPTTVRSNSSKLD

SEQ ID NO: 14 - protein, 649 aa, Plasmodium falciparum
DYIKGDPYFAEYATKLSFILNSSDANTSSGETANHNDEACNCNESEISSVEHASISDPSSNKTCNTHSSIKANKKKVCKHVKLGVRENDKDLRVCVIEHTSLSGVENCCFKDFLRILQENCSDNKSGSSSNGSCDKNNEEACEKNLEKVFASLTNCYKCEKCKSEQSKKNNKKWTWRKSSGNKEGLQEEYANTIGLPPRTQSLCLVVCLDEKEGKKTQELKNIRTNSELLKEWIIAAFHEGKNLKPSHEKKNDDNGKKNDDNNSKLCKDLKYSFADYGDLIKGTSIWDNEYTKDLELNLQKIFGKLFRKYIKKNIASDENTLYSSLDELRESWWNTNKKYIWLAMKHGAEMNGTTCNADGSVTGSGSSCDDIPTIDLIPQYLRFLQEWVEHFCKQRQAKVKDVIENCKSCKESGNKCKTECKNKCEAYKKFIENCKGGDGTAGSSWVKRWDQIYMRYSKYIEDAKRNRKAGTKNCGPSSITNVSASTDENKCVQSDIDSFFKHLIDIGLTTPSSYLSIVLDDNICGDDKAPWTTYTTYTTYTTYTTYTTTKNCDKERDKSKSQSCNTAVVVNVPSPLGNTPHEYKYACECRTPSNKELCDDRKEYMNQWSSGSAQTVRDRSGKDYYELYTYNGVKETKLPKKLNSSKLD

SEQ ID NO: 15 - protein, 632 aa, Plasmodium falciparum; identical to SEQ ID NO: 13

SEQ ID NO: 16 - protein, 643 aa, Plasmodium falciparum
SYVKDDPYSAEYVTKLSFILNSSDANTSSETPSKYYDEVCNCNESEISSVGQAQTSGPSSNKTCITHSSIKTNKKKVCKDVKLGINNNDKVLRVCVIEDTSLSGVDNCCCQDLLGILQENCSDKNQSGSSSNGSCNNKNQDECQKKLEKVFASLTNGYKCDKCKSGTSRSKKKWIWRKSSGNEEGLQKEYANTIGLPPRTQSLYLGNLPKLENVCKGVTDIIYDTKEKFLSGCLIAAFHEGKNLKTSHEKKNDDNGKKLCKALEYSFADYGDLIKGTSIWDNDFTKDLELNLQKIFGKLFRKYIKKNNTAEQDTSYSSLDELRESWWNTNKKYIWTAMKHGAGMNSTTCSGDGSVTGSGSSCDDMPTIDLIPQYLRFLQEWVEHFCKQRQEKVKDVITNCNSCKECGDTCNGECKTECKTKCKGECEKYKNFIEECNGTADGGTSGSSWSKRWDQIYKRYSKYIEDAKRNRKAGTKNCGTSSTTNAAASTTENKCVQSDIDSFFKHLIDIGLTTPSSYLSNVLDDNICGEDKAPWTTYTTYTTKNCDIQKKTPKPQSCDTLVVVNVPSPLGNTPHGYKYVCECKIPTTEETCDDRKEYMNQWIIDTSKKQKGSGSTNNDYELYTYNGVQIKQAAGTLKNSKLD

SEQ ID NO: 17 - protein, 631 aa, Plasmodium falciparum
DYIKGDPYFAEYATKLSFILNSSDANNPSEKIQKNNDEVCNCNESGISSVEQASISDPSSNKTCNTHSSIKTNKKKECKHVKLGVRENDKVLKICVIEDTSLSGVENCCFKDLLGILQEPRIDKNQSGSSSNGSCDKNSEEICQKKLDEALASLHNGYKCDKCKSGTSTVNKNWIWKKFPGNGEGLQKEYANTIGLPPRTHSLYLGNLPKLENVCEDVKDINFDTKEKFLAGCLIAAFHEGKNLKTTYPQNKKKLCKALKYSFADYGDLIKGTSIWDNDFTKDLELNLQKAFGKLFRKYIKKNIASDENTSYSSLDELRESWWNTNKKYIWLAMKHGAGMNITTCNADGSVTGSGSSCDDIPTIDLIPQYLRFLQEWVEHFCEQRQAKVKDVIKNCNSCKESGGTCNSDCEKKCKIECEKYKKFIEECRTAAEGTAGSSWVKRWDQIYMRYSKYIEDAKRNRKAGTKNCGTSSTTNAAASKCVQSDIDSFFKHLIDIGLTTPSSYLSIVLDENNCGADKAPWTTYTTYTTTKNCDIQKDKSKSQSCDTLVVVNVPSPLGNTPHGYKYACQCKIPTTEESCDDRKEYMNQWIIDTSKKQKGSGSTNNDYELYTYNGVKETKLPKKSSSSKLD

SEQ ID NO: 18 - protein, 628 aa, Plasmodium falciparum
NYIKGDPYFAEYATKLSFILNSSDTENASETPSKYYDEACNCNESEIASVGQAQTSGPSSNKTCITHSSIKTNKKKECKDVKLGINNNDKVLRVCVIEDTSLSGVDNCCCQDLLGILQENCSDNKRGSSSNGSCDKNSEEICQKKLEKVFASLTNGYKCDKCKSGTSRSKKKWIWKKSSGNEEGLQKEYANTIGLPPRTQSLCLVCLHEKEGKTQHKTISTNSELLKEWIIAAFHEGKNLKTSHEKKNDDNGKKLCKALEYSFADYGDLIKGTSIWDNEYTKDLELNLQKIFGKLFRKYIKKNNTAEQHTSYSSLDELRESWWNTNKKYIWTAMKHGAGMNGTTCSCSGDSSNDMPTIDLIPQYLRFLQEWVEHFCKQRQEKVNAVIENCNSCKESGGTCNSDCKTECKNKCEAYKEFIEDCKGGGTGTAGSPWSKRWDQIYKRYSKHIEDAKRNRKAGTKNCGTSSTTNAAASTDENKCVQSDVDSFFKHLIDIGLTTPSSYLSNVLDDNICGADKAPWTTYTTYTTTKNCDIQKKTPKSQSCDTLVVVNVPSPLGNTPHEYKYACECKIPTTEETCDDRKEYMNQWSCGSAQTVRGRSGKDDYELYTYNGVKETKPLGTLKNSKLD

SEQ ID NO: 19 - protein, 628 aa, Plasmodium falciparum
DYIKDDPYSAQYTTKLSFILNPSDANTSSEKIQKNNDEACNCNESGISSVGQAQTSGPSSNKTCITHSSIKANKKKVCKDVKLGINNNDKVLRVCVIEDTSLSGVDNCCCQDLLGILQENCSDNKRGSSSNGSCNNNNEEACEKNLDEAPASLHNGYKNQKCKSGTSRSKKKWIWKKSSGNEKGLQEEYANTIGLPPRTQSLCLVCLHEKEGKTQHKTISTNSELLKEWIIAAFHEGKNLKTSHEKKNDDNGKKLCKALEYSFADYGDLIKGTSIWDNEYTKDLELNLQKAFGKLFRKYIKKNNTAEQDTSYSSLDELRESWWNTNKKYIWIAMKHGAGMNGTTCSCSGDSSNDMPTIDLIPQYLRFLQEWVEHFCEQRQAKVKDVITNCKSCKESGNKCKTECKTKCKDECEKYKTFIEDCNGGGTGTAGSSWVKRWDQIYKRYSKHIEDAKRNRKAGTKNCGPSSITNAAASTDENKCVQSDIDSFFKHLIDIGLTTPSSYLSNVLDENSCGDDKAPWTTYTTYTTTKNCDIQKDKSKSQPINTSVVVNVPSPLGNTPYRYKYACECKIPTTEESCDDRKEYMNQWSCGSARTMKRGYKNDNYELCKYNGVDVKPTTVRSNSSKLD

SEQ ID NO: 20 - protein, 637 aa, Plasmodium falciparum
NYIKDDPYSKEYVTKLSFIPNSSDANTSSEKIQKNNDEVCNPNESGISSVEQAQTSDPSSNKTCITHSSIKANKKKECKDVKLGVRENDKDLKICVIEHTSLSGVDNCCFKDFLRMLQEPRIDKNQRGSSSNGSCDKNSEEACEKNLDEALASLTNGYKCDKCKSEQSKKNNNKWIWKKFPGKEGGLQEEYANTIGLPPRTQYLCLVVCLDEKEGKTQELKNIRTNSELLKEWIIAAFHEGKNLKTTYPQKKNDDNGKKLCKDLKYSFADYGDLIKGTSIWDNEYTKNVELNLQNNFGKLFRKYIKKNNTAEQDTSYSSLDELRESWWNTNKKYIWLAMKHGAEMNSTTCCGDGSVTGSGSSCDDIPTIDLIPQYLRFLQEWVEHFCKQRQAKVKDVITNCNSCKESGNKCKTECKNKCKDECEKYKKFIEACGTAVGGTGTAGSPWSKRWDQIYKRYSKHIEDAKRNRKAGTKNCGPSSTTNAAENKCVQSDIDSFFKHLIDIGLTTPSSYLSIVLDDNICGADKAPWTTYTTYTTENCDIQKKTPKSQSCDTLVVVNVPSPLGNTPHGYKYACQCRTPNKQESCDDRKEYMNQWIIDNTKNPKGSGSGKDYYELCKYNGVKETKPLGTLKNSKLD

SEQ ID NO: 21 - protein, 639 aa, Plasmodium falciparum
DYIKGDPYSAEYVTKLSFIPNSSDANNPSEKIQKNNDEVCNCNESEISSVGQASISDPSSNKTCNTHSSIKANKKKVCKDVKLGVRENDKVLKICVIEHTSLRGVDNCCFKDLLGILQEPRIDKNQSGSSSNGSCDKNSEEACEKNLEKVLASLTNGYKCDKCKSGTSRSKKKWIWKKYSGKEGGLQEEYANTIGLPPRTQSLCLVVCLDEKEGKTQELKNISTNSELLKEWIIAAFPEGKNLKPSPEKKKGDNGKKLCKDLKYSFADYGDLIKGTSIWDNEYTKDLELNLQKIFGKLFRKYIKKNIASDENTLYSSLDELRESWWNTNKKYIWLAMKHGAGMNSTMCNADGSVTGSGSSCDDMPTIDLIPQYLRFLQEWVEHFCKQRQEKVKPVIENCNSCKNTSSERKIGGTCNSDCKTECKNKCEVYKKFIEDCKGGDGTAGSSWSKRWDQIYKRYSKYIEDAKRNRKAGTKNCGPSSTTNAAENKCVQSDIDSFFKHLIDIGLTTPSSYLSTVLDDNICGEDNAPWTTYTTYTTTKNCDKDKKKSKSQSCDTLVVVNVPSPLGNTPHEYKYACECRTPNKQESCDDRKEYMNQWISDNTKNPKGSGSGKDYYELYTYNGVDVKPTTVRSSSTKLD

SEQ ID NO: 22 - protein, 646 aa, Plasmodium falciparum
DYIKDDPYSKEYTTKLSFILNSSDANTSSEKIQKNNDEVCNPNESEISSVEQAQTSRPSSNKTCITHSSIKANKKKVCKDVKLGVRENDKVLRVCVIEHTSLSGVENCCCQDLLGILQENCSDNKRGSSSNGSCDKNSEEACEKNLDEALASLTNCYKNQKCKSEQSKKNNNKWIWKKSSGKEGGLQKEYANTIGLPPRTQSLYLGNLPKLENVCKGVTDINFDTKEKFLAGCLIAAFHEGKNLKTTYLEKKNDDNGKKLCKALEYSFADYGDLIKGTSIWDNEYTKDLELNLQKAFGKLFRKYIKKNNTAEQDTSYSSLDELRESWWNTNKKYIWTAMKHGAGMNGTTCSSGSGDSSNDIPTTDFIPQYLRFLQEWVENFCEQRQAKVKDVIENCNSCKNTSGERKIGDTCNSDCEKKCKDECEKYKKFIEDCKGGDGTAGSSWVKRWDQIYKRYSKHIEDAKRNRKAGTKNCGITTGTISGESSGATSGVTTTENKCVQSDIDSFFKHLIDIGLTTPSSYLSNVLDDNICGEDNAPWTTYTTYTTEKCNKETDKSKSQQSNTAVVVNVPSPLGNTPHGYKYACECKIPTTEETCDDRKEYMNQWSCGSAQTVRDRSGKDDYELCKYNGVQIKQAAGTLKNSKLD

SEQ ID NO: 23 - protein, 642 aa, Plasmodium falciparum
YIKNNPYSSEDGKLLIFDNTNAFIESPTYYNNVCCCSTPEKSAKTDGSSSSSSFGTSFSYENSVTSNKGKECKQIKFSGNKNNMNINICSPPDEKLLVKLEDLLKGFCDTCDPDIGVEVVSEENCEEQYKKLLPSLEKCTILTCKECNKTRCKPLKKVEEKWIWKKSSGNGEGLQKEYANTIGLPPRTQSLYLGNLPKLENVCKGVTDINFDTKEKFLAGCLIAAFHEGKNLKTSPEKKKGENKRKLCKALEYSFADYGDLIKGTSIWDNEYTKDLELNLQNNFGKLFRKYIKKNISTEQHTSYSSLDELRESWWNTNKKYIWTAMKHGAEMNGTTCSSGSGDNGDSSITGSSDSGSTTCSGDNGSISCDDIPTIDFIPQYLRFLQEWVEHFCKQRQAKVNAVITNCKSCKESGDTCNSDCEKKCKIECEKYKTFIEECGTAAGGTAGSPWSKRWDQIYKRYSKYIEDAKRNRKAGTKNCGPSSTTSTAESKCVQSDIDSFFKHLIDIGLTTPSSYLSIVLDDNICGADKAPWTTYTTYTTTEKCNKERDKSKSQSSDTLVVVNVPSPLGNTPHGYKYACQCKIPTTEETCDDRKEYMNQWISDTSKNPKGSGSTNNDYELYTYTGSEVKMSQKKLNSPKLD

SEQ ID NO: 24 - protein, 640 aa, Plasmodium falciparum
SYVKNDPYSKEYVTKLSFILNPSDANNPSGETANHNDEACNPNESEIASVGQAQTSDRLSQKACITHSFIGANKKIVCKDVKLGVREKDKDLKICVIEDDSLRGVENCCFKDLLGILQENCSDNKSGSSSNGSCNNKNQDECQKKLDEALASLHNGYKCDKCKSGTSRSKKIWTWRKFPGNGEGLQKEYANTIGLPPRTQSLYLGNLRKLENVCKGVTDINFDTKEKFLAGCLIAAFHEGKNLKISNKKKNDDNGKKLCKDLKYSFADYGDLIKGTSIWDNEYTKDLELNLQKIFGKLFRKYIKKNIASDENTLYSSLDELRESWWNTNKKYIWLAMKHGTTCSSGSGDNGDGSVTGSGSSCDDMSTIDLIPQYLRFLQEWVEHFCKQRQEKVKDVIENCKSCKNTSGERIIGGTCGSDCKTKCKGECDAYKNFIEECKRGDGTAGSPWSKRWDQIYMRYSKYIEDAKRNRKAGTKNCGTSSTTNAAENKCVQSDIDSFFKHLIDIGLTTPSSYLSIVLDENICGDDKAPWTTYTTYTTTEKCNKETDKSKSQSCNTAVVVNVPSPLGNTPHGYKYACECKIPTTEETCDDRKEYMNQWISDTSKKPKGGRSTNNDYELYTYNGVKETKLPKKSSSSKLD

SEQ ID NO: 25 - protein, 643 aa, Plasmodium falciparum
DYIKDDPYSKEYTTKLSFILNSSDANTSSGETANHNDEACNCNESEISSVGQAQTSGPSSNKTCITHSFIKANKKKVCKDVKLGVRENDKVLRVCVIEDTSLSGVDNCCCQDLLGILQENCSDNKRGSSSNGSCNNKNQDECQKKLEKVFVSLTNGYKCDKCKSGTSTVNKKWIWKKSSGNEKGLQKEYANTIGLPPRTQSLYLGNLPKLGNVCEDVTDINFDTKEKFLAGCLIAAFHEGKNLKISHEKKKGDNGKKLCKALEYSFADYGDLIKGTSIWDNEYTKDLELNLQKAFGKLFGKYIKKNIASDENTSYSSLDELRESWWNTNKKYIWTAMKHGAEMNSTMCNADGSVTGSGSSCDDIPTTDFIPQYLRFLQEWVEHFCKQRQEKVNAVIENCNSCKNTSGERKIGGTCNGDCKTECKNKCEAYKNFIEDCKGGDGTAGSSWVKRWDQIYKRYSKHIEDAKRNRKAGTKSCGPSSITNASVSTDENKCVQSDIDSFFKHLIDIGLTTPSSYLSIVLDENNCGEDNAPWTTYTTYTTTEKCNKDKKKSKSQSCNTAVVVNVPSPLGNTPHEYKYACQCKIPTTEETCDDRKEYMNQWISDTSKKQKGSGSTNNDYELYTYTGVKETKLPKKLNSPKLD

SEQ ID NO: 26 - protein, 656 aa, Plasmodium falciparum
DYIKGDPYFAEYATKLSFILNSSDANNPSGETANHNDEVCNPNESEISSVGQAQTSDPSSNKTCNTHSSIKANKKKVCKHVKLGINNNDKVLRVCVIEDTSLSGVENCCFKDLLGILQENCSDNKSGSSSNGSCNNKNQEACEKNLEKVLASLTNCYKCDKCKSGTSTVNKNWIWKKSSGNKEGLQKEYANTIGLPPRTHSLYLGNLPKLENVCEDVKDINFDTKEKFLAGCLIAAFHEGKNLKKRYPQNKNDDNNSKLCKALEYSFADYGDLIKGTSIWDNEYTKDLELNLQQIFGKLFRKYIKKNISTEQDTLYSSLDELRESWWNTNKKYIWLAMKHGAGMNITTCCGDGSVTGSGSSCDDIPTIDLIPQYLRFLQEWVEHFCKQRQEKVKDVINSCNSCKNTSSKTKLGDTCNSDCEKKCKIECEKYKKFIEECRTAVGGTAGSSWSKRWDQIYKMYSKHIEDAKRNRKAGTKNCGITTGTISGESSGANSGVTTTENKCVQSDIDSFFKHLIDIGLTTPSSYLSIVLDDNICGDDKAPWTTYTTYTTYTTTEKCNKERDKSKSQQSNTSVVVNVPSPLGNTPHGYKYACQCKIPTNEETCDDRKEYMNQWISDTSKNPKGSGSTNNDYELYTYNGVKETKLPKKLNSPKLD

SEQ ID NO: 27 - protein, 647 aa, Plasmodium falciparum
DYIKDDPYSAEYATKLSFILNPSDANTSSGETANHNDEVCNCNESEIASVELAPISDSSSNKTCITHSFIGANKKKECKDVKLGVREKDKDLKICVIEDDSLRGVENCCCQDLLGILQENCSDNKSGSSSNGSCDKNSEDECQKKLENVFASLKNGYKCDKCKSGTSTVNKKWIWRKYSGNGEGLQKEYANTIGLPPRTHSLYLVCLHEKEGKTQHKTISTNSELLKEWIIAAFHEGKNLKTSHQNNNSGNKKKLCKALKYSFADYGDLIKGTSIWDNDFTKDLELNLQKIFGKLFRKYIKKNIASDENTSYSSLDELRESWWNTNKKYIWLAMKHGAEMNSTMCNGDGSVTGSSDSGSTTCSGDNGSISCDDIPTIDLIPQYLRFLQEWVEHFCKQRQEKVKDVITNCKSCKESGDTCNSDCEKKCKNKCEAYKKFIEERRTAAQGTAESSWVKRWDQIYMRYSKYIEDAKRNRKAGTKSCGPSSTTNAAASTAENKCVQSDIDSFFKHLIDIGLTTPSSYLSIVLDDNICGADNAPWTTYTTYTTTKNCDIKKKTPKPQSCDTLVVVNVPSPLGNTPHEYKYACQCRTPNKQESCDDRKEYMNQWSSGSAQTVRGRSTNNDYELYTYNGVKETKPLGTLKNSKLD

SEQ ID NO: 28 - protein, 632 aa, Plasmodium falciparum; identical to SEQ ID NO: 9

SEQ ID NO: 29 - protein, 632 aa, Plasmodium falciparum; identical to SEQ ID NO: 9

SEQ ID NO: 30 - protein, 649 aa, Plasmodium falciparum; identical to SEQ ID NO: 14

SEQ ID NO: 31 - protein, 644 aa, Plasmodium falciparum
NYIKGDPYSAEYATKLSFILNSSDTENASEKIQKNNDEVCNCNESEIASVEQAQTSGSSSNKTCITHSSIKANKKKECKDVKLGINNNDKDLKICVIEDTSLSGVDNCCFKDFLRILQENCSDNKRGSSSNGSCNNNNEEICQKKLEKVLASLTNGYKCDKCKSGTSTVNKNWIWKKSSGNGEGLQKEYANTIGLPPRTQSLCLVCLHEKEGKTQELKNISTNSELLKEWIIAAFHEGKNLKTSHQKKNDDNGKKLCKALEYSFADYGDLIKGTSIWDNEYTKDLELNLQKIFGKLFRKYIKKNNTIVENTSYSSLDELRESWWNTNKKYIWTAMKHGAGMNGTTCSSGDNGDSSNDIPTTDFIPQYLRFLQEWVEHFCEQRQGKVKHVMESCKSCKNTSSKTKLGGKCGNDCEKKCKDECEKYKTFIEECVTAAGGTAGSPWSKRWDQIYKRYSKYIEDAKRNRKAGTKNCGTSSTTNAAASTAESKCVQSDIDSFFKHLIDIGLTTPSSYLSIVLDENNCGEDKAPWTTYTTYTTYTTYTTTKNCDKDKKKSKSQPINTSVVVNVPSPLGNTPHGYKYACQCKIPTTEESCDDRKEYMNQWISDTSKNPKGSRSTNNDYELYTYNGVQIKQAAGRSSSTKLD

SEQ ID NO: 32 - protein, 672 aa, Plasmodium falciparum
NYIKGDPYFAEYATKLSFILNPSDANTSSEKIQKNNDEACNCNESGISSVGQAPISDPSSNKTCNTHSSIKTNKKKVCKDVKLGINNNDKVLRVCVIEDDSLRGVDNCCFKDLLGILQENCSDKNQSGSSSNGSCDKNSEEICQTKLEKVLASLTNCYKCDKCKSGTSRSRKIWTWRKFRGNGEGLQKEYANTIGLSPRTQSLCLVVCLDEKEGKTQHKTISTNSELLKEWIIAAFHEGKNLKKRYPQNKNDDNGKKNDDNNSKLCKDLKYSFADYGDLIKGTSIWDNEYTKNVELNLQKIFGKLFRKYIKKNISTEQDTSYSSLDELRESWWNTNKKYIWLAMKHGAEMNGTTCSCSGDSSSGENQTNSCDDIPTIDLIPQYLRFLQEWVEHFCKQRQEKVKDVIENCNSCKECGGTCNGECKTECEKKCKNKCEAYKNFIEVCTGGDGTAGSSWVKRWDQIYMRYSKYIEDAKRNRKAGTKNCGTSSTTNVSVSAAENKCVQSDIDSFFKHLIDIGLTTPSSYLSIVLDENNCGDDKAPWTTYTTYTTYTTYTTYTTYTTYTTYTTYTTTKKCNKETDKSKSQSCNTAVVVNVPSPLGNTPHGYKYACECRTPNKQETCDDRKEYMNQWIIDTSKNPKGSGSGKDYYELYTYNGVQIKQAAGRSNNSKLD

SEQ ID NO: 33 - protein, 655 aa, Plasmodium falciparum
SYVKNDPYFAEYATKLSFIPNSSDTENASEKIQKNNDEVCNPNESEIACVELAQTSDSSSQKACITHSFIKANKKKECKDVKLGINNNDKDLKICVIEHTSLSGVENCCCQDLLGMLQENCSDKNQSGSSSNGSCDKNNEDECQKKLEKVLASLTNCYKNQKCKSGTSTVNKNWIWKKYSGTEGGLQKEYANTIALPPRTQSLCLVCLHEKEEKTQELKNISTNSELLKEWIIAAFHEGKNLKKRYHQNNNSGNKKKLCKALKYSFADYGDLIKGTSIWDNDFTKNLELNLQKIFGKLFRKYIKKNISTEQHTSYSSLDELRESWWNTNKKYIWTAMKHGAGMNGTTCCGDGSVTGSSDSGSTTCCGDGSVTGSGSSCDDIPTIDLIPQYLRFLQEWVEHFCEQRQAKVKDVIKNCNSCKECGGTCNGECKTECEKKCKGECEAYKKFIEKCNGGGGEGTSGSSWSKRWDQIYMRYSKYIEDAKRNRKAGTKNCGTSSTTNAAENKCVQSDIDSFFKHLIDIGLTTPSSYLSIVLDENICGEDKAPWTTYTTYTTEKCNKETDKSKSQSCDTLVVVNVPSPLGNTPHGYKYACQCRTPSNKELCDDRKEYMNQWISDNTKNPKGSGSGKDDYELYTYNGVQIKQAAGRSSSTKLD

SEQ ID NO: 34 - protein, 630 aa, Plasmodium falciparum
NYIKGDPYSKEYVTKLSFILNPSDANNPSGETANHNDEVCNPNESGIASVEHAQTSGSSSNKTCITHSSIKTNKKKVCKHVKLGVRENDKDLKICVIEDTSLSGVENCCCQDLLGILQENCSDNKRRSSSNGSCDNKNQDECEKNLEKVLASLTNCYKCDKCKSGTSTVNNKWIWKKSSGKEGGLQKEYANTIGLPPRTQSLYLGNLPKLENVCEDVTDINFDTKEKFLAGCLIAAFHEGKNLKTTYLEKKNADNNSKLCKALEYSFADYGDLIKGTSIWDNEYTKDLELNLQNNFGKLFRKYIKKNIASDENTLYSSLDELRESWWNTNKKYIWLAMKHGAGMNGTTCSSGSGDNGSISCDDIPTIDLIPQYLRFLQEWVEHFCKQRQAKVKDVIKNCNSCKESGNKCKTECKNKCEAYKKFIEEFCTAAGGTSGSPWSKRWDQIYKMYSKYIEDAKRNRKAGTKNCGTSSTTSTAESKCVQSDIDSFFKHLIDIGLTTPSSYLSIVLDENNCGDDKAPWTTYTTYTTTKNCDKDKKKSKSQSCNTAVVVNVPSPLGNTPHGYKYACECKIPTTEESCDDRKEYMNQWISDTSKKQKGSGSGKDYYELYTYNGVDVKPTTVRSSSSKLD

SEQ ID NO: 35 - protein, 653 aa, Plasmodium falciparum
DYIKGDPYFAEYATKLSFILNPSDTENASETPSKYYDEACNPNESEIASVEQAQTSGPSSNKTCITHSSIKTNKKKECKDVKLGVRENDKDLKICVIEDTSLSGVDNCCFKDLLGILQENCSDNKRGSSSNDSCNNNNEEACEKNLDEALASLTNGYKCDKCKSGTSTVNKKWTWRKSSGNEEGLQKEYANTIGLPPRTQSLCLVCLHEKEGKTKHKTISTNSELLKEWIIAAFHEGKNLKTSHEKKNDDNGKKLCKALEYSFADYGDLIKGTSIWDNEYTKDLELNLQKAFGKLFRKYIKKNNTAEQDTSYSSLDELRESWWNTNKKYIWTAMKHGAEMNGTTCSSGSGDNGDSSITGSSDSGSTTCSGDNGSISCDDIPTTDFIPQYLRFLQEWVEHFCEQRQAKVKDVINSCNSCNESGGTCNGECKTKCKDECEKYKKFIEDCNGGDGTAGSSWVKRWDQIYKRYSKHIEDAKRNRKAGTKNCGPSSITNAAASTDENKCVQSDVDSFFKHLIDIGLTTPSSYLSIVLDENSCGDDKAPWTTYTTYTTTEKCNKERDKSKSQSSDTLVVVNVPSPLGNTPHEYKYACECKIPTNEETCDDRKDYMNQWISDTSKKQKGSGSGKDYYELYTYNGVQIKQAAGRSSSTKLD

SEQ ID NO: 36 - protein, 662 aa, Plasmodium falciparum
DYIKDDPYFAEYVTKLSFILNSSDANTSSGETANHNDEVCNCNESEISSVEQEQISGPSSNKTCNTHSSIKANKKKVCKHVKLGVREKDKDLKICVIEDTSLSGVDNCCFKDLLGILQENCSDNIRESSSNGSCNNNNEEICQKKLDEALASLTNGYKCEKCKSGTSRSKKNWIWKKSSGNGEGLQKEYANTIGLPPRTHSLYLGNLPKLENVCEDVTDINFDTKEKFLAGCLIAAFHEGKNLKISNKNKNDDNNSKLCKALEYSFADYGDLIKGTSIWDNEYTKDLELNLQKIFGKLFRKYIKKNNTAEQDTSYSSLDELRESWWNTNKKYIWTAMKHGAEMNSTTCCGDGSVTGSSDSGSTTCSGDNGSISCDDMSTIDLIPQYLRFLQEWVEHFCEQRQAKVKDVIENCNSCKECGGTCNGECKTECKNKCKDECEKYKKFIEECRTAAEGTAESSWVKRWDQIYKRYSKYIEDAKRNRKAGTKNCGITTGTISGESSGANSGVTTTESKCVQSDIDSFFKHLIDIGLTTPSSYLSIVLDENNCGEDNAPWTTYTTYTTTKNCDIQKKTPKSQSCNTAVVVNVPSPLGNTPHGYKYACQCKIPTTEESCDDRKEYMNQWSCGSAQTVRGRSTNNDYELCKYNGVKETKPLGTLKNSKLN

SEQ ID NO: 37 - protein, 590 aa, Plasmodium falciparum
DYIKGDPYSKEYGKLLKFDNTNAFIESPTYYNNVCCCSTPEKSAKTDGSSCSSSFGTQDNNLLVEFQELLKSFCDTCDTDIGVEVVCENNCEEQYKKLLPSLEKCTILTCNECNKTRCKPLKKVEEKWIWKKYSGKEGGLQKEYANTIGLPPRTQSLCLVCLHEKEGKTQHKTISTNSELLKERIIAAFHEGKNLKTSHENKNDDNGKKLCKALKYSFADYGDLIKGTSIWDNEYTKDLELNLQKIFGKLFRKYIKKNISTEQHTLYSSLDELRESWWNTNKKYIWTAMKHGAEMNGTTCCGDGSVTGSGSSCDDIPTIDLIPQYLRFLQEWVEHFCKQRQEKVNAVITNCNSCKECGGTCNGECKTECKTKCKVACDAYKEFIEKCVSAAGGTSGSSWSKRWDQIYKRYSKYIEDAKRNRKAGTKSCGTSSTTSTAENKCVQSDIDSFFKHLIDIGLTTPSSYLSIVLDENNCGEDKAPWTTYTTYTTTKNCDKEKDKSKSQSCNTAVVVNVPSPLGNTPHEYKYVCECRTPNKQESCDDRKEYMNQWIIDNTKNPKGSGSTNNDYELCKYNGVKETKPLGTLKNSKLD

SEQ ID NO: 38 - protein, 643 aa, Plasmodium falciparum
DYIKNDPYSAEYATKLSFILNSSDSNNASKIIPNHIDEASNCNESMISSATQASILDPSSQKVCNTHSFIGANKKKECKVIKLGVNNNDRILRVCVIEDTSLSGVASCCCQDLLGIVKELCKDNKERETRSSDNCDKNNQDECQKKLEEVLSCLQNGYKCEKCKLSTQKKCDNKWIWKIFTGEGGGLQEEYANTIGLPQRTQSLCLGNLYGEGEKKEENRNINSNTELLKEWIIASFHEGKILKTCYPQNNSGDNKKKLCKALEYSFADYGDLIKGTSIWDNEYTKDLELNLQKTFGKLFRKYIKRNISSEQNSLYDSLAELRESWWNTNKKYIWIAMKYGAGMKSTTCNGGNCGDNGSSCDDMPTIDLIPQYLRFLQEWVEHFCKQRQEKVNDVITNCKSCKESGGKCNGDCKNKCKVECEKYKTFIDGTGSGTAGSTWSKRWDQIYKRYSKHIEDAKRNLEAGTKTCGTSSGVNRATNTAASSGTTSDASKCLQSDIDSFFKHLVDIGLTTPSSYLSNVLDENNCGADKAPWTIYTTYTTTTKDKCAKVKLKSQPSDSTVVVNVPSPLGNTPHGYKYVCECRTPTNKELCDDRKEYMNQWNCDNTQNSKVARSRNNDYESCKYNGVKETKPSGTLKNSKLN

SEQ ID NO: 39 - protein, 666 aa, Plasmodium falciparum
DNYVKEFFKNFKGDNYKSLDDYIKGDPYSAEYATKLSFILNPSDANTSSGETANHNDEACNCNESEIASVGQAQISDRLSQKACNTHSFIGANKKKECKDVKLGVHENDKVLRVCVIEDDSLRGVDNCCCQDFLRMLQENCSDNKRESSSNGSCDKNNEEACEKNLEKVFASLTNGYKCDKCKSEQSKKNNKNWIWKKYSGNGEGLQKEYANTIGLPPRTHSLYLGNLRKLENVCEDVKDINFDTKEKFLAGCLIAAFHEGKNLKTSHEKKKGDNGKKLCKDLKYSFADYGDLIKGTSIWDNEYTKDLELNLQQIFGKLFRKYIKKNNTIVENTSYSSLDELRESWWNTNKKYIWLAMKHGAEMNSTTCNADGSVTGSGSSCDDIPTIDLIPQYLRFLQEWVEHFCEQRQAKVNAVITNCKSCKESGGTCGSDCKTKCKDECEKYKNFIEECRTAADGTAGSSWSKRWDQIYKMYSKHIEDAKRNRKAGTKNCGITTGTISGESSGANSGVTTTENKCVQSDIDSFFKHLIDIGLTTPSSYLSIVLDENNCGEDKAPWTTYTTYTTTKNCDKEKDKSKSQSCNTAVVVNVPSPLGNTPHEYKYACQCKIPTNEETCDDRKEYMNQWSSGSAQTVRGRSTNNDYELYTYNGVQIKPTTVRSSSTKLD

SEQ ID NO: 40 - protein, 611 aa, Plasmodium falciparum
DYIKDDPYFAEYVTKLSFILNSSDTENASEKIQKNNDEACNSNESGISSVGQAQTSCPSSNKTCITHSSIKANKKKVCKDVKLGVRENDKVLRVCVIEHTSLSGVENCCCQDLLGILQEPRIDKNQKCKSEQSKKNNNKWIWKKYSGKEGGLQKEYANTIGLPPRTQSLYLGNLPKLENVCKDVTDINFDTKEKFLAGCLIAAFHEGKNLKTTYPQNKNAENKKKLCKDLKYSFADYGDLIKGTSIWDNDFTKDLELNLQKAFGKLFRKYIKKNISTEQHTLYSSLDELRESWWNTNKKYIWTAMKHGAEMNITTCCGDGSVTGSGSSCDDMPTTDFIPQYLRFLQEWVEHFCKQRQAKVNAVIENCNSCKNTSSKTKLGGKCGSDCEKKCKVACDAYKTFIEECGTAVGGTAGSSWVKRWDQIYKRYSKHIEDAKRNRKAGTKNCGTSSTTNAAASTAENKCVQSDIDSFFKHLIDIGLTTPSSYLSIVLDDNNCGEDKAPWTTYTTYTTTKNCDIQKDKSKSQSCDTLVVVNVPSPLGNTPHEYKYACQCKIPTTEESCDDRKEYMNQWSCGSAQTVRGRSGKDYYELCKYNGVKETKLPKKLNSPKLD

SEQ ID NO: 41 - protein, 656 aa, Plasmodium falciparum
DYIKDDPYSAQYVTKLSFILNPSDTENASETPSKYYDEVCNPNESGIASVEHAQTSDSSSQKACNTHSSIKTNKKKVCKHVKLGVRENDKDLKICVIEHTSLSGVENCCCQDLLGILQENCSDNKRRSSSNGSCDNKNQDECEKNLEKVLASLTNCYKCDKCKSGTSTVNNKWIWKKYSVKEGGLQKEYANTIALPPRTQSLYLVCLHEKEGKTQELKNIRTNSELLKEWIIAAFHEGKNLKISPQNKNDDNGKKLCKALKYSFADYGDLIKGTSIWDNDFTKDLELNLQKIFGKLFRKYIKKNISTEQDTLYSSLDELRESWWNTNKKYIWTAMKHGAEMNGTTCCGDGSVTGSSDSGSTTCSGDNGSISCDDIPTIDLIPQYLRFLQEWVEHFCKQRQENVNAVIENCNSCKESGGTCNSDCEKKCKIECEKYKNFIEECNGTAAGGTSGSSWSKRWDQIYKRYSKYIEDAKRNRKAGTKNCGITTGTISGESSGATSGVTTTENKCVQSDIDSFFKHLIDIGLTTPSSYLSIVLDDNICGEDKAPWTTYTTYTTKNCDKEKDKSKSQSCNTAVVVNVPSPLGNTPHGYKYACECKIPTTEETCDDRKEYMNQWSSGSAQTVRDRSGKDDYELYTYNGVKETKLPKKSSSTKLD

SEQ ID NO: 42 - protein, 658 aa, Plasmodium falciparum
NYIKGDPYFAEYATKLSFILNSSDTENASEKIQKNNDEVCNCNESEIASVEQEQISGPSSNKTCNTHSSIKTNKKKECKHVKLGINNNDKDLKICVIEDDSLRGVENCCFKDFLRILQENCSDNKRESSSNGSCNNKNQEACEKNLDEALASLTNCYKCEKCKSGTSTVNKNWIWKKSSGDEKGLQKEYANTIGLPPRTHSLYLGNLPKLENVCEDVTDINFDTKEKFLAGCLIAAFHEGKNLKKRYPQNKNDDNNSKLCKDLKYSFADYGDLIKGTSIWDNEYTKDLELNLQKAFGKLFGKYIKKNNTAEQDTSYSSLDELRESWWNTNKKYIWLAMKHGTTCSSGTCDNGDGSVTGSSDSGSTTCSGDNGSISCDDMPTIDLIPQYLRFLQEWVEHFCKQRQAKVKDVIKNCNSCKNTSGERIIGGTCGSDCKTKCKVACDAYKKFIEKCGTAADGTAGSSWSKRWDQIYKMYSKHIEDAKRNRKAGTKNCGPSSTTNVSVSTDENKCVQSDIDSFFKHLIDIGLTTPSSYLSIVLDENICGEDKAPWTTYTTYTTKNCDKEKDKSKSQSCNTAVVVNVPSPLGNTPHGYKYACQCKIPTTEETCDDRKEYMNQWIIDTSKKQKGSGSTNNDYELYTYTGSEVKMSQKKLNSPKLD

SEQ ID NO: 43 - protein, 656 aa, Plasmodium falciparum; identical to SEQ ID NO: 41

SEQ ID NO: 44 - protein, 658 aa, Plasmodium falciparum
DYIKGDPYFAEYATKLSFILNSSDANTSSEKIQKNNDEVCNCNESGISSVGQAQTSCPSSNKTCITHSSIKANKKKECKDVKLGVREKDKVLKICVIEDDSLRGVENCCFKDLLGILQENCSDNKRESSSNGSCNNKNQDECQKKLEKVFASLTNCYKCEKCKSGTSRSKKIWIWKKYSGNGEGLQKEYANTIGLPPRTQSLCLVVCLDEKGKKTQELKNIRTNSELLKEWIIAAFHEGKNLKTTYPQKKNDDNNSKLCKDLKYSFADYGDLIKGTSIWDNDFTKDLELNLQKIFGKLFRKYIKKNNTIVENTSYSSLDELRESWWNTNKKYIWTAMKHGAGMNSTMCNADGSVTGSSDSGSTTCSGDNGSGSSCDDIPTIDLIPQYLRFLQEWVEHFCKQRQEKVNAVITNCKSCKESGGTCNSDCKTECKNKCEAYKNFIEDCKGGGTGTAGSSWVKRWYQIYMRYSKYIEDAKRNRKAGTKSCGTSSGANSGVTTTENKCVQSDIDSFFKHLIDIGLTTPSSYLSIVLDENICGADKAPWTTYTTYTTYTTYTTTKNCDKDKKKSKSQSCDTLVVVNVPSPLGNTPHGYKYACECKIPTNEETCDDRKEYMNQWISDTSKNPKGGRSTNNDYELYTYNGVKETKPLGTLKNSKLN

SEQ ID NO: 45 - protein, 658 aa, Plasmodium falciparum
NYIKGDPYFAEYATKLSFILNSSDTENASEKIQKNNDEVCNCNESEIASVEQEQISGPSSNKTCNTHSSIKTNKKKECKHVKLGINNNDKDLKICVIEDDSLRGVENCCFKDFLRILQENCSDNKRESSSNGSCNNKNQEACEKNLDEALASLTNCYKCEKCKSGTSTVNKNWIWKKSSGDEEGLQEEYANTIGLPPRTHSLYLGNLPKLENVCEDVTDINFDTKEKFLAGCLIAAFHEGKNLKKRYPQNKNDDNNSKLCKDLKYSFADYGDLIKGTSIWDNEYTKDLELNLQKAFGKLFGKYIKKNNTAEQDTSYSSLDELRESWWNTNKKYIWLAMKHGTTCSSGSGDNGDGSVTGSSDSGSTTCSGDNGSISCDDMPTIDLIPQYLRFLQEWVEHFCKQRQAKVKDVIKNCNSCKNTSGERIIGGTCGSDCKTKCKVACDAYKKFIEKCGTAADGTAGSSWSKRWDQIYKMYSKHIEDAKRNRKAGTKNCGPSSTTNVSVSTDENKCVQSDIDSFFKHLIDIGLTTPSSYLSIVLDENICGEDKAPWTTYTTYTTKNCDKEKDKSKSQSCNTAVVVNVPSPLGNTPHGYKYACQCKIPTTEETCDDRKEYMNQWIIDTSKKQKGSGSTNNDYELYTYTGSEVKMSQKKLNSPKLD

SEQ ID NO: 46 - protein, 633 aa, Plasmodium falciparum
DYIKGDPYSKEYVTKLSFILNSSDANTSSEKIQKNNDEVCNCNESEISSVEQAQTSDPSSNKTCITHSSIKANKKKVCKHVKLGVRENDKDLRVCVIEHTSLSGVENCCFKDFLRILQENCSDNKSGSSSNGSCNNKNQEACEKNLEKVLASLTNCYKCDKCKSEQSKKNNKNWIWKKSSGKEGGLQKEYANTIGLPPRTQSLCLVVCLDEKGKKTQELKNIRTNSELLKEWIIAAFHEGKNLKPSHEKKNDDNGKKLCKALEYSFADYGDLIKGTSIWDNEYTKDLELNLQKIFGKLFRKYIKKNNTAEQDTSYSSLDELRESWWNTNKKYIWLAMKHGAGMNSTTCCGDGSVTGSGSSCDDIPTIDLIPQYLRFLQEWVEHFCKQRQEKVKPVIENCKSCKESGGTCNGECKTECKNKCEVYKKFIEECGTAAGGTAGSPWSKRWDQIYKRYSKHIEDAKRNRKAGTKNCGPSSTTNAAENKCVQSDIDSFFKHLIDIGLTTPSSYLSIVLDDNICGADKAPWTTYTTYTTTEKCNKETDKSKSQSCNTAVVVNVPSPLGNTPHGYKYACQCKIPTNEETCDDRKEYMNQWSCGSARTMKRGYKNDNYELCKYNGVDVKPTTVRSNSSKLD

SEQ ID NO: 47 - protein, 648 aa, Plasmodium falciparum
SYVKNNPYSSEDGKLLKFDNTNAFKESITCNKNVCSCSGNEKLIISEGSLSSSSFGTSSSYQSSIITSKKRNECAQIKFSGNENNMNIKICSTQDNNLLVKLEDLLKGFCDTCDTGIGVEVVSENNCEEQYKKLLPSLEKCTVLNCNECNKTRCKPLKKQQEKWIWGKPKQEAAGLQEEYANTIGLPPRTQSLYLGNLRKLENVSKGVTDINFDTKEKFLAGCLIAAFHEGKNLKTSHENKNDDNGKKLCKDLKYSFADYGDLIKGTSIWDNEYTKDLELNLQKAFGKLFRKYIKKNNTAEQDTSYSSLDELRESWWNTNKKYIWLAMKHGAGMNGTTCCGDGSVTGSSDSGSTTCCGDGSVTGSGSSCDDIPTIDLIPQYLRFLQEWVEHFCEQRQAKVKDVIKNCKSCKNTSGERKIGDTCGNDCEKKCKVACDAYKEFIEECRTAAEGTAGSSWVKRWDQIYKRYSKYIEDAKRNRKAGTKNCGPSSTTNAAESKCVQSDIDSFFKHLIDIGLTTPSSYLSIVLDENNCGEDNAPWTTYTTYTTTKNCDIQKKTPKSQSCNTAVVVNVPSPLGNTPHGYKYACECKIPTTEETCDDRKEYMNQWISDNTKNPKGSGSTNNDYELYTYNGVKETKLPKKSSSSKLD

SEQ ID NO: 48 - protein, 670 aa, Plasmodium falciparum
NYIKDDPYFAEYATKLSFIPNSSDANNPSETPSKYYDEACNPNESEIACVGQAQTSGPSSNKTCITHSSIKTNKKKVCKHVKLGINNNDKDLKICVIEDTSLSGVENCCFKDFLRMLQENCSDNKRESSSNGSCNNKNQDECQKKLDEALASLTNGYKCEKCKSEQSKKNKKIWTWKKSSGNKEGLQEEYANTIGLSPRTQSLCLVCLHEKEGKTQELKNISTNSELLKEWIIAAFHEGKNLKPSHENKNDNGKKLCKDLKYSFADYGDLIKGTSIWDNEYTKDLELNLQKIFGKLFRKYIKKNNTIVENTSYSSLDELRESWWNTNKKYIWLAMKHGAGMNSTTCNADGSVTGSSDSGSTTCCGDGSVTGSGSSCDDIPTIDLIPQYLRFLQEWVEHFCEQRQAKVKDVIENCKSCKNTSGERKIGGTCGSDCKTKCKNKCDAYKKFIDGTGSGGGSRPTGTAGSSWSKRWDQIYMRYSKYIEDAKRNRKAGTKSCGITTGTISGESSGANSGVTTTESKCVQSDIDSFFKHLIDIGLTTPSSYLSNVLDENNCGEDKAPWTTYTTYTTTKNCDKDKKKSKSQPINTSVVVNVPSPLGNTPHGYKYACECKIPTTEETCDDRKEYMNQWSRGSAQTVRGRSTNNDYELYTYNGVQIKQAAGTLNSPKLD

SEQ ID NO: 49 - protein, 630 aa, Plasmodium falciparum
SYVKNNPYSSEDGKLLKFDNTNAFKESITCNKNVCSCSGNEKLIISEGSSSSSSFGTSFSYENSVTSNKRKECKQIKFSGNKNNMNIKICSTQDNNLLVKLEDLLKGFCDTCDTDIGVEVVSENNCEEQYKKLLPCLEKCTVLNCNECNKTVFKNLKKQQEKWIWGKPKQEAAGLQKEYANTIGLPPRTQSLYLGNLPKLGNVCKGVTDINFDTKEKFLAGCLIAAFHEGKNLKTTYPQNKKKLCKDLKYSFADYGDLIKGTSIWDNEYTKDLELNLQKAFGKLFRKYIKKNISTEQHTLYSSLDELRESWWNTNKKYIWTAMKHGAEMNSTMCNADGSVTGSGSSCDDIPTIDLIPQYLRFLQEWVEHFCKQRQEKVNAVINSCNSCKNTSSKTKLGGKCGSDCEKKCKIECEKYKKFIEEYVTAVGGTSGSPWSKRWDQIYKRYSKYIEDAKRNRKAGTKSCGTSSTTNAAASTAESKCVQSDIDSFFKHLIDIGLTTPSSYLSIVLDDNICGADNAPWTTYTTYTTTKNCDKDKKKSKSQQSNTAVVVNVPSPLGNTPHGYKYACQCKIPTTEETCDDRKEYMNQWISDTSKKQKGSGSTNNDYELYTYNGVKETKPLGTLKNSKLD

SEQ ID NO: 50 - protein, 651 aa, Plasmodium falciparum
NYIKDDPYSKEYVTKLSFILNSSDTENASEKIQKNNDEVCNPNESGISSVEQAQTSDPSSNKTCNTHSFIGANKKKECKDVKLGINNNDKVLKICVIEDDSLRGVENCCFKDLLGILQENCSDNKSGSSSNGSCDNKNQEACEKNLEKVLASLTNCYKCDKCKSEQSKKNNNIWIWRKSSGKEGGLQKEYANTIGLPPRTQSLCLVVCLDEKGKKTQELKNIRTNSELLKEWIIAAFHEGKNLKPSLEKKKGDNNSKLCKDLKYSFADYGDLIKGTSIWDNEYTKNVELNLQNNFGKLFRKYIKKNIASDENTSYSSLDELRESWWNTNKKYIWTAMKHGAGMNGTMCNADGSVTGSGSSCDDIPTIDLIPQYLRFLQEWVEHFCKQRQEKVKPVIENCKSCKNTSSKTKLGGTCNGECKTECKNKCEAYKTFIEEFRTAAGGTAGSPWSKRWDQIYKMYSKHIEDAKRNRKAGTKNCGITTGTISGESSGATSGVTTTESKCVQSDIDSFFKHLIDIGLTTPSSYLSIVLDENNCGEDNAPWTTYTTYTTKNCDKEKDKSKSQSCNTAVVVNVPSPLGNTPHGYKYACQCKIPTTEESCDDRKEYMNQWIIDNTKNPKGSGSTNNDYELYTYNGVQIKQAAGRSSSTKLD

SEQ ID NO: 51 - protein, 611 aa, Plasmodium falciparum
SYVKNNPYSAEYGKLLKFDGPDAFIESPTYYNNVCCCSTPEKSAKTHGSSSSSSFGTSFSYENSVTSNKRKECKQIKFSGNKNNMNINICSTQDEKLLVKLEDLLKGFCDTCDTDIGVEVVCEENCEEQFKKLLPSLEKCTILTCKECNKTRCKPLKKVEEKWIWKKSSGNEKGLQKEYANTIGLPPRTQSLCLVCLHEKEGKTQHKTISTNSELLKEWIIAAFHEGKNLKTTYPQNKNDDNNSKLCKALEYSFADYGDLIKGTSIWDNEYTKDLELNLQKAFGKLFRKYIKKNNTAEQHTSYSSLDELRESWWNTNKKYIWTAMKHGAGMNGTTCSCSGDSSNDIPTTDFIPQYLRFLQEWVENFCEQRQAKVKDVINSCNSCKESGGTCGSDCEKKCKDECEKYKTFIEEFCTAAGGTSGSPWSKRWDQIYKRYSKDIEDAKRNRKAGTKNCGTSTAENKCVQSDIDSFFKHLIDIGLTTPSSYLSIVLDENNCGDDKAPWTTYTTYTTTKNCDKDKKKSKLQQCNTAVVVNVPSPLGNTPHGYKYACECKIPTTEESCDDRKEYMNQWSSGSAQTVRDRSGKDDYELYTYNGVDVKPTTVRSSSTKLD

SEQ ID NO: 52 - protein, 633 aa, Plasmodium falciparum; identical to SEQ ID NO: 46

SEQ ID NO: 53 - protein, 630 aa, Plasmodium falciparum
DYIKGDPYSSEDGKLLIFDNTNAFIESPTYYNNVCCCSTPEKSAKTDGSSCSSSFGTSFSYQSSIITSKKRNECAQIKFSGNKNNMNINICSTQDNNLLVEFQELLKGFCDTCDTDIGVEVVCENNCEEQYKKLLPCLEKCTVLNCNECNKTRCKPLKKEQEKWIWKKYSGKEGGLQKEYANTIGLPPRTQSLCLVCLHEKEGKTQHKTISTNSELLKEWIIDAFHEGKNLKTTYPQKKNADNGKKLCKALKYSFADYGDLIKGTSIWDNDFTKDLELNLQKIFGKLFRKYIKKNISTEQHTLYSSLDELRESWWNTNKKYIWTAMKHGAGMNGTTCSCSGDSSSGENQTNSCDDIPTIDLIPQYLRFLQEWVEHFCEQRQGKVKDVIKNCKSCKECGGTCNGECKTECKTKCKGECEKYKEFIEECKGKAAEGTSGSSWVKRWDQIYKRYSKYIEDAKRNRKAGTKSCGTSSTTNAAENKCVQSDIDSFFKHLIDIGLTTPSSYLSIVLDDNICGADNAPWTTYTTYTTKNCDIQKDKSKSQSCNTAVVVNVPSPLGNTPHEYKYACECRTPNKQESCDDRKEYMNQWISDTSKNPKGGRSTNNDYELCKYNGVDVKPTTVRSSSSKLD

SEQ ID NO: 54 - protein, 633 aa, Plasmodium falciparum
DYIKGDPYSKEYVTKLSFILNSSDANTSSEKIQKNNDEVCNCNESEISSVEQAQTSDPSSNKTCITHSSIKANKKKVCKHVKLGVRENDKDLRVCVIEHTSLSGVENCCFKDFLRILQENCSDNKSGSSSNGSCNNKNQEACEKNLEKVLASLTNCYKCDKCKSEQSKKNNKNWIWKKSSGKEGGLQKEYANTIGLPPRTQSLCLVVCLDEKGKKTQELKNIRTNSELLKEWIIAAFHEGKNLKPSHEKKNDDNGKKLCKALEYSFADYGDLIKGTSIWDNEYTKDLELNLQKIFGKLFRKYIKKNNTAEQDTSYSSLDELRESWWNTNKKYIWLAMKHGAGMNSTTCCGDGSVTGSGSSCDDIPTIDLIPQYLRFLQEWVEHFCKQRQEKVKPVIENCKSCKESGGTCNGECKTECKNKCEVYKKFIEELWTAAGGTAGSPWSKRWDQIYKRYSKHIEDAKRNRKAGTKNCGPSSTTNAAENKCVQSDIDSFFKHLIDIGLTTPSSYLSIVLDDNICGADKAPWTTYTTYTTTEKCNKETDKSKSQSCNTAVVVNVPSPLGNTPHGYKYACQCKIPTNEETCDDRKEYMNQWSCGSARTMKRGYKNDNYELCKYNGVDVKPTTVRSNSSKLD

SEQ ID NO: 55 - protein, 634 aa, Plasmodium falciparum
NYIKDDPYSKEYVTKLSFIPNSSDANNPSGETANHNDEVCNPNESEISSVEHAQTSVLLSQKAYITHSSIKANKKKVCKYVKLGVRENDKDLKICVIEDDSLRGVENCCFKDFLRILQENCSDNKRESSSNGSCNNNNEEACEKNLDEALASLTNCYKNQKCKSGTSTVNNKWIWKKSSGKEGGLQKEYANTIALPPRTQSLCLVVCLDEKGKKTQELKNISTNSELLKERIIASFHEGKNLKTSHEKKNADNRKKNADNNSKLCKALKYSFADYGDLIKGTSIWDNEYTKDLELNLQNNFGKLFRKYIKKNNTAEQHTSYSSLDELRESWWNTNKKYIWLAMKHGAGMNGTTCSSGSGDSSNDIPTTDFIPQYLRFLQEWVEHFCKQRQEKVNAVIENCKSCKESGNKCKTECEKKCEAYKKFIEKCNGGAAEGTSGSSWSKRWDQIYMRYSKYIEDAKRNRKAGTKNCGPSSGANSGVTTTENKCVQSDIDSFFKHLIDIGLTTPSSYLSIVLDENICGADNAPWTTYTTYTTEKCNKETDKSKPQSCNTAVVVNVPSPLGNTPHGYKYACQCRTPSNKELCDDRKEYMNQWSSGSAQTVRDRSGKDYYELCKYNGVKETKLPKKSSSSKLD

SEQ ID NO: 56 - protein, 651 aa, Plasmodium falciparum
NYIKGDPYFAEYATKLSFILNSSDTENASETPSKYYDEACNCNESGIACVGQAQTSDRLSQKACNTHSFIGANKKKECKDVKLGVRENDKDLKICVIEHTSLSGVENCCCQDLLGILQENCSDKNQSGSSSNGSCDKNSEEACEKNLDEALASLTNGYKCEKCKSEQSKKNNKIWTWRKFPGNGEGLQKEYANTIGLSPRTQLLYLVCLHEKGKKTQELKNIRTNSELLKEWIIAAFHEGKNLKKRYLEKKKGDNNSKLCKDLKYSFADYGDLIKGTSIWDNDFTKDLELNLQQIFGKLFRKYIKKNNTAEQDTLYSSLDELRESWWNTNKKYIWTAMKHGAGMNSTTCCGDGSVTGSSDSGSTTCSGDNGSISCDDIPTIDLIPQYLRFLQEWVEHFCKQRQAKVKDVITNCKSCKESGGTCNSDCKTKCKGECEKYKTFIEHCKGVGGTGTAGSSWVKRWYQIYMRYSKYIEDAKRNRKAGTKSCGTSSGANSGVTTTESKCVQSDIDSFFKHLIDIGLTTPSSYLSIVLDENICGDDKAPWTTYTTYTTKNCDKDKKTPKPQQSNTAVVVNVPSPLGNTPHGYKYACQCKIPTTEETCDDRKEYMNQWSSGSAQTVRDRSTNNDYELYTYNGVQIKQAAGTLNSSKLD

SEQ ID NO: 57 - protein, 650 aa, Plasmodium falciparum
SYVKNDPYSAEYATKLSFILNSSDANTSSGETANHNDEVCNCNESEISSVELAPISGPSSNKTCNTHSSIKTNKKKECKHVKLGVREKDKDLKICVIEDTSLSGVENCCFKDFLRMLQENCSDNIRGSSSNGSCDKNSEEACEKNLEKVFASLTNGYKCDKCKSGTSTVNNKWIWKKYSGKEGGLQKEYANTIALPPRTQSLCLVVCLDEKEGKTQELKNIRTNSELLKEWIIAAFHEGKNLKTTYPQNKNAENKKKLCKALKYSFADYGDLIKGTSIWDNDFTKDLELNLQQIFGKLFRKYIKKNNTIVENTSYSSLDELRESWWNTNKKYIWTAMKHGAEMNGTMCNADGSVTGSSDSGSTTCSGDNGSISCDDMPTIDLIPQYLRFLQEWVEHFCKQRQEKVNAVITNCKSCKESGGTCGSDCKTKCKGECEAYKTFIEKCNGTAAEGTSGSPWSKRWYQIYMRYSKYIEDAKRNRKAGTKNCGTSSGATSGVTTTENKCVQSDIDSFFKHLIDIGLTTPSSYLSIVLDDNICGADKAPWTTYTTYTTKNCDIQKDKSKLQQCNTAVVVNVPSPLGNTPHGYKYACQCRTPSNKESCDDRKEYMNQWSCGSAQTVRGRSTNNDYELYTYNGVKETKPLGTLKNSKLN

SEQ ID NO: 58 - protein, 653 aa, Plasmodium falciparum
DYIKGDPYFAEYVTKLSFILNSSDTENASEKIQKNNDEACNCNESEISSVEQEQISGSSSNKTCNTHSSIKANKKKECKDVKLGVREKDKVLRVCVIEDDSLRGVENCCCQDLLGMLQENCSDNKSGSSSNDSCDKNNEDECQKKLEKVFASLTNGYKCEKCKSEQSKKNNNKWIWRKFPGNGEGLQKEYANTIGLPPRTHSLYLGNLPKLENVCEDVTDINFDTKEKFLAGCLIAAFHEGKNLKTTYLEKKKGDNGKKLCKALKYSFADYGDLIKGTSIWDNEYTKDLELNLQKIFGKLFRKYIKKNNTAEQHTSYSSLDELRESWWNTNKKYIWLAMKHGAEMNGTMCNADGSVTGSGSSCDDIPTIDLIPQYLRFLQEWVEHFCEQRQGKVKHVMESCKSCKNTSGERKIGGTCNGDCKTECKNKCDAYKTFIEECRTAAEGTAESSWSKRWDQIYKRYSKYIEDAKRNRKAGTKNCGITTGTISGESSGANSGVTTTENKCVQSDIDSFFKHLIDIGLTTPSSYLSIVLDDNICGEDNAPWTTYTTYTTTKICDKDKKKSKSQSCNTAVVVNVPSPLGNTPHEYKYACECRTPTTEESCDDRKEYMNQWSCGSAQTVRGRSTNNDYELYTYNGVKETKPLGTLKNSKLN

SEQ ID NO: 59 - protein, 611 aa, Plasmodium falciparum
DYIKDDPYFAEYVTKLSFILNSSDTENASEKIQKNNDEACNSNESGISSVGQAQTSCPSSNKTCITHSSIKANKKKVCKDVKLGVRENDKVLRVCVIEHTSLSGVENCCCQDLLGILQEPRIDKNQKCKSEQSKKNNNKWIWKKYSGKEGGLQKEYANTIGLPPRTQSLYLGNLPKLENVCKDVTDINFDTKEKFLAGCLIAAFHEGKNLKTTYPQNKNAENKKKLCKDLKYSFADYGDLIKGTSIWDNDFTKDLELNLQKAFGKLFRKYIKKNISTEQHTLYSSLDELRESWWNTNKKYIWTAMKHGAEMNITTCCGDGSVTGSGSSCDDMPTTDFIPQYLRFLQEWVEHFCKQRQAKVNAVIENCNSCKNTSSKTKLGGKCGSDCEKKCKVACDAYKTFIEECGTAGGGTAGSSWVKRWDQIYKRYSKHIEDAKRNRKAGTKNCGTSSTTNAAASTAENKCVQSDIDSFFKHLIDIGLTTPSSYLSIVLDDNNCGEDKAPWTTYTTYTTTKNCDIQKDKSKSQSCDTLVVVNVPSPLGNTPHEYKYACQCKIPTTEESCDDRKEYMNQWSCGSAQTVRGRSGKDYYELCKYNGVKETKLPKKLNSPKLD

SEQ ID NO: 60 - protein, 623 aa, Plasmodium falciparum
DYIKDDPYSAEYGKLLKFDNTNAFKESITCNKNVCSCSGNEKLIISEGSSSSCSFGTSSSYQSSIITSNKRKECKQIKFSGNKNNMNINICSTQDEKLLVKLEELLKSFCNTCDIGIGVEVVCENNCEEQYKKLLPCLEKCTVLNCNECNKTRCKPLKKEQEKWIWKKYSVKEGGLQEEYANTIALPPRTQSLCLVCLHEKEEKTQELKNISTNSELLKERIIAAFHEGKNLKTTYPQNNNSGNKENLCKALKYSFADYGDLIKGTSIWDNDFTKDLELNLQKAFGKLFRKYIKKNIASDENTSYSSLDELRESWWNTNKKYIWLAMKHGAGMNGTTCCGDGSVTGSGSSCDDIPTIDLIPQYLRFLQEWVEHFCEQRQEKVKHVMESCKSCKECGGTCGSDCEKKCKAYKEFIEKCKGQAAEGTSGSSWSKRWDQIYKRYSKYIEDAKRNRKAGTKNCGPSSTTNAAASTTENKCVQSDIDSFFKHLIDIGLTTPSSYLSIVLDDNICGADKAPWTTYTTYTTEKCNKETDKSKSQSCDTAVVVNVPSPLGNTPHEYKYACQCRTPSNKELCDDRKEYMNQWSSGSAQTVRDRSTNNDYELYTYNGVQIKQATGTLKNSKLD

SEQ ID NO: 61 - protein, 650 aa, Plasmodium falciparum
SYVKNNPYSAEYVTKLSFILNSSDANTSSETPSKYYDEVCNCNESEISSVGQAQTSGPSSNKTCITHSSIKTNKKKVCKDVKLGINNNDKVLRVCVIEDTSLSGVDNCCCQDLLGILQENCSDKNQSGSSSNGSCNNKNQDECQKKLEKVFASLTNGYKCDKCKSGTSRSKKKWIWRKSSGNEEGLQKEYANTIGLPPRTQSLYLGNLRKLENVCKGVTDINFDTKEKFLAGCLIAAFHEGKNLKTTYPQNKKKLCKDLKYSFADYGDLIKGTSIWDNEYTKDLELNLQKAFGKLFRKYIKKNISTEQHTLYSSLDELRESWWNTNKKYIWLAMKHGAGMNSTTCCGDGSVTGSGSSCDDIPTIDLIPQYLRFLQEWVEHFCKQRQEKVNAVIENCNSCKECGDTCNGECKTECEKKCKIECEKYKTFIEECVTAVGGTSGSPWSKRWDQIYKRYSKYIEDAKRNRKAGTKNCGITTGTISGESSGANSGVTTTENKCVQSDIDSFFKHLIDIGLTTPSSYLSIVLDDNICGADNAPWTTYTTYTTYTTTKNCDIKKKTPKSQPINTSVVVNVPSPLGNTPHGYKYACQCKIPTTEESCDDRKEYMNQWIIDTSKKQKGSGSTNNDYELYTYNGVKETKLPKKSSSSKLD

SEQ ID NO: 62 - protein, 652 aa, Plasmodium falciparum
DYIKDDPYFAEYVTKLSFILNSSDANNPSGETANHNDEVCNPNESGIASVEQAQTSDPSSNKTCNTHSSIKANKKKVCKHVKLGVRENDKDLKICVIEHTSLSGVENCCCQDFLRILQENCSDNKSGSSSNGSCNNKNQEACEKNLEKVLASLTNCYKCDKCKSEQSKKNNKNWIWKKSSGNEKGLQKEYANTIGLPPRTQSLCLVVCLDEKEGKTQELKNIRTNSELLKEWIIAAFHEGKNLKKRYPQNKNDDNNSKLCKDLKYSFADYGDLIKGTSIWDNEYTKDLELNLQNNFGKLFRKYIKKNISTEQDTLYSSLDELRESWWNTNKKYIWLAMKHGAGMNSTTCSSGSGSTTCSSGSGSTTCSSGSGDSCDDMPTTDFIPQYLRFLQEWVEHFCKQRQEKVNAVIKNCNSCKESGGTCNGECKTECKNKCEAYKTFIEEFCTADGGTSGSPWSKRWDQIYKMYSKHIEDAKRNRKAGTKNCGPSSTTNVSVSTDENKCVQSDIDSFFKHLIDIGLTTPSSYLSIVLDDNICGEDKAPWTTYTTYTTTKKCNKETDKSKSQSCNTAVVVNVPSPLGNTPHGYKYACECKIPTTEETCDDRKEYMNQWIIDTSKKQKGSGSGKDDYELYTYNGVDVKPTTVRSNSTKLD

SEQ ID NO: 63 - protein, 667 aa, Plasmodium falciparum
SYVKNNPYSKEYVTKLSFILNPSDANNPSETPSKYYDEVCNCNESGIACVGQAQTSGPSSNKTCITHSFIGANKKKVCKDVKLGVREKDKDLKICVIEDTYLSGVDNCCFKDFLGMLQENCSDNKSGSSSNGSCNNKNQDECEKNLDEALASLTNGYKCEKCKSGTSTVNKYWIWRKSSGNKEGLQKEYANTIALPPRTHSLCLVVCLDEKEGKTQHKTISTNSELLKEWIIAAFHEGKNLKTSHEKKKGDDGKKNADNNSKLCKALKYSFADYGDLIKGTSIWDNDFTKDLELNLQKIFGKLFRKYIKKNIASDENTSYSSLDELRESWWNTNKKYIWLAMKHGAGMNSTTCCGDGSVTGSSDSGSTTCCGDGSVTGSGSSCDDMPTTDFIPQYLRFLQEWVEHFCKQRQENVNAVIENCNSCKECGGTCNSDCEKKCKTECKGECDAYKEFIEKCNGGAAEGTSGSSWSKRWDQIYKRYSKYIEDAKRNRKAGTKNCGTSSTTSTAESKCVQSDIDSFFKHLIDIGLTTPSSYLSIVLDENICGADNAPWTTYTTYTTYTTYTTTEKCNKETDKSKLQQCNTSVVVNVPSPLGNTPHGYKYVCECRTPNKQETCDDRKEYMNQWISDNTKNPKGSRSTNNDYELYTYNGVQIKPTTVRSNSTKLD

SEQ ID NO: 64 - protein, 709 aa, Plasmodium falciparum; identical to SEQ ID NO: 11

SEQ ID NO: 65 - protein, 697 aa, Plasmodium falciparum
MSAWSHPQFEKGGGSGGGSGGSAWSHPQFEKGSAGSAAGSGEFSYVKNNPYSAEYGKLLIFDNTNAFKESITFNKNVCSCSGNEKLIISEGSSSSSSFGTSSSYQSSIITSKKRNECAQIKFSGNENNMNINICSTQDEKLLVKLEDLLKGFCNISGVNTGGVEVVSEENCEEQFKKLLPSLEKCTILTCKECNKTRCKPLKKVEEKWIWRKFPGNGEGLQKEYANTIGLPPRTQSLYLGNLPKLENVCEDVKDINFDTKEKFLAGCLIAAFHEGKNLKKRYPQNKNDDNGKKLCKALEYSFADNGDLIKGTSIWDNEYTKDLELNLQKAFGKLFGKYIKKNNTAEQHTSYSSLDELRESWWNTNKKYIWLAMKHGAEMNGTTCSCSGDSSNDMPTIDLIPQYLRFLQEWVEHFCKQRQAKVKPVIENCKSCKESGGTCNGECKTECKNKCEAYKNFIEDCKRGDGTAGSSWSKRWDQIYKRYSKHIEDAKRNRKAGTKNCGPSSITNAAASTDESKCVQSDIDSFFKHLIDIGLTTPSSYLSIVLDENNCGDDKAPWTTYTTTKNCDIQKKTPKPQQSDTSVVVNVPSPLGNTPYRYKYACQCKIPTTEESCDDRKEYMNQWSCGSAQTVRGRSGKDYYELCKYNGVQIKPTTVRSNSTKLDGGADYKDHDGDYKDHDIDYKDDDDKGGSHHHHHH

SEQ ID NO: 66 - protein, 711 aa, Plasmodium falciparum
MSAWSHPQFEKGGGSGGGSGGSAWSHPQFEKGSAGSAAGSGEFDINYIKGDPYFAEYATKLSFILNSSDANNPSEKIQKNNDEVCNCNESGIASVEQEQISDPSSNKTCITHSSIKANKKKVCKHVKLGVRENDKDLRVCVIEHTSLSGVENCCCQDFLRILQENCSDNKSGSSSNGSCNNKNQEACEKNLEKVLASLTNCYKCDKCKSEQSKKNNKNWIWKKSSGKEGGLQKEYANTIGLPPRTQSLCLVVCLDEKGKKTQELKNIRTNSELLKEWIIAAFHEGKNLKPSHEKKNDDNGKKLCKALEYSFADYGDLIKGTSIWDNEYTKDLELNLQKIFGKLFRKYIKKNNTAEQDTSYSSLDELRESWWNTNKKYIWLAMKHGAGMNSTTCCGDGSVTGSGSSCDDIPTIDLIPQYLRFLQEWVEHFCKQRQEKVKPVIENCKSCKESGGTCNGECKTECKNKCEVYKKFIEDCKGGDGTAGSSWVKRWDQIYKRYSKYIEDAKRNRKAGTKNCGPSSTTNAAENKCVQSDIDSFFKHLIDIGLTTPSSYLSIVLDDNICGADKAPWTTYTTYTTTEKCNKETDKSKLQQCNTAVVVNVPSPLGNTPHGYKYACQCKIPTNEETCDDRKEYMNQWSCGSARTMKRGYKNDNYELCKYNGVDVKPTTVRSNSSKLDGGADYKDHDGDYKDHDIDYKDDDDKGGSHHHHHH

SEQ ID NO: 67 - protein, 728 aa, Plasmodium falciparum
MSAWSHPQFEKGGGSGGGSGGSAWSHPQFEKGSAGSAAGSGEFDIDYIKGDPYFAEYATKLSFILNSSDANTSSGETANHNDEACNCNESEISSVEHASISDPSSNKTCNTHSSIKANKKKVCKHVKLGVRENDKDLRVCVIEHTSLSGVENCCFKDFLRILQENCSDNKSGSSSNGSCDKNNEEACEKNLEKVFASLTNCYKCEKCKSEQSKKNNKKWTWRKSSGNKEGLQEEYANTIGLPPRTQSLCLVVCLDEKEGKKTQELKNIRTNSELLKEWIIAAFHEGKNLKPSHEKKNDDNGKKNDDNNSKLCKDLKYSFADYGDLIKGTSIWDNEYTKDLELNLQKIFGKLFRKYIKKNIASDENTLYSSLDELRESWWNTNKKYIWLAMKHGAEMNGTTCNADGSVTGSGSSCDDIPTIDLIPQYLRFLQEWVEHFCKQRQAKVKDVIENCKSCKESGNKCKTECKNKCEAYKKFIENCKGGDGTAGSSWVKRWDQIYMRYSKYIEDAKRNRKAGTKNCGPSSITNVSASTDENKCVQSDIDSFFKHLIDIGLTTPSSYLSIVLDDNICGDDKAPWTTYTTYTTYTTYTTYTTTKNCDKERDKSKSQSCNTAVVVNVPSPLGNTPHEYKYACECRTPSNKELCDDRKEYMNQWSSGSAQTVRDRSGKDYYELYTYNGVKETKLPKKLNSSKLDGGADYKDHDGDYKDHDIDYKDDDDKGGSHHHHHH